European Patent Specification EP 3 751 000 B1, published November 27, 2024. Title: Adeno-associated viral vector with hepatocyte growth factor for treatment of eye diseases. Applicant: NIPPON MEDICAL SCHOOL FOUNDATION TEIKA PHARMACEUTICAL CO., LTD. Application JP2018-019963. The sequence listing filed with the application follows.

SEQUENCE LISTING (16 sequences)

SEQ ID NO: 1 - DNA, 930 bp, Cytomegalovirus
aatcaatattggccattagccatattattcattggttatatagcataaatcaatattggctattggccattgcatacgttgtatccatatcataatatgtacatttatattggctcatgtccaacattaccgccatgttgacattgattattgactagttattaatagtaatcaattacggggtcattagttcatagcccatatatggagttccgcgttacataacttacggtaaatggcccgcctggctgaccgcccaacgacccccgcccattgacgtcaataatgacgtatgttcccatagtaacgccaatagggactttccattgacgtcaatgggtggagtatttacggtaaactgcccacttggcagtacatcaagtgtatcatatgccaagtacgccccctattgacgtcaatgacggtaaatggcccgcctggcattatgcccagtacatgaccttatgggactttcctacttggcagtacatctacgtattagtcatcgctattaccatggtgatgcggttttggcagtacatcaatgggcgtggatagcggtttgactcacggggatttccaagtctccaccccattgacgtcaatgggagtttgttttggcaccaaaatcaacgggactttccaaaatgtcgtaacaactccgccccattgacgcaaatgggcggtaggcgtgtacggtgggaggtctatataagcagagctcgtttagtgaaccgtcagatcgcctggagacgccatccacgctgttttgacctccatagaagacaccgggaccgatccagcctccgcggccgggaacggtgcattggaacgcggattccccgtgccaagagtgacgtaagtaccgcctatagagtctataggcccacccccttggcttcttatgcatgctatactgtttttggcttg

SEQ ID NO: 2 - DNA, 344 bp, Artificial Sequence
  CMV promoter for p42 (p42CMV)
attatgcccagtacatgaccttatgggactttcctacttggcagtacatctacgtattagtcatcgctattaccatggtgatgcggttttggcagtacatcaatgggcgtggatagcggtttgactcacggggatttccaagtctccaccccattgacgtcaatgggagtttgttttggcaccaaaatcaacgggactttccaaaatgtcgtaacaactccgccccattgacgcaaatgggcggtaggcgtgtacggtgggaggtctatataagcagagctcgtttagtgaaccgtcagatcgcctggagacgccatccacgctgttttgacctccatagaaga

SEQ ID NO: 3 - DNA, 584 bp, Artificial Sequence
  CMV promoter for p13 (p13CMV)
attaatagtaatcaattacggggtcattagttcatagcccatatatggagttccgcgttacataacttacggtaaatggcccgcctggctgaccgcccaacgacccccgcccattgacgtcaataatgacgtatgttcccatagtaacgccaatagggactttccattgacgtcaatgggtggagtatttacggtaaactgcccacttggcagtacatcaagtgtatcatatgccaagtacgccccctattgacgtcaatgacggtaaatggcccgcctggcattatgcccagtacatgaccttatgggactttcctacttggcagtacatctacgtattagtcatcgctattaccatggtgatgcggttttggcagtacatcaatgggcgtggatagcggtttgactcacggggatttccaagtctccaccccattgacgtcaatgggagtttgttttggcaccaaaatcaacgggactttccaaaatgtcgtaacaactccgccccattgacgcaaatgggcggtaggcgtgtacggtgggaggtctatataagcagagctcgtttagtgaaccgtcagatc

SEQ ID NO: 4 - DNA, 2187 bp, Artificial Sequence
  Codon optimized human HGF (optHGF) gene sequence
atgtgggtgaccaagctgctgcccgccctgctgctgcagcacgtgctgctgcacctgctgctgctgcccatcgccatcccctacgccgagggccagcggaagcggcggaacaccatccacgagttcaagaagagcgccaagaccaccctgatcaagatcgaccccgccctgaagatcaagaccaagaaggtgaacaccgccgaccagtgcgccaaccggtgcacccggaacaagggcctgcccttcacctgcaaggccttcgtgttcgacaaggcccggaagcagtgcctgtggttccccttcaacagcatgagcagcggcgtgaagaaggagttcggccacgagttcgacctgtacgagaacaaggactacatccggaactgcatcatcggcaagggccggagctacaagggcaccgtgagcatcaccaagagcggcatcaagtgccagccctggagcagcatgatcccccacgagcacagcttcctgcccagcagctaccggggcaaggacctgcaggagaactactgccggaacccccggggcgaggagggcggcccctggtgcttcaccagcaaccccgaggtgcggtacgaggtgtgcgacatcccccagtgcagcgaggtggagtgcatgacctgcaacggcgagagctaccggggcctgatggaccacaccgagagcggcaagatctgccagcggtgggaccaccagaccccccaccggcacaagttcctgcccgagcggtaccccgacaagggcttcgacgacaactactgccggaaccccgacggccagccccggccctggtgctacaccctggacccccacacccggtgggagtactgcgccatcaagacctgcgccgacaacaccatgaacgacaccgacgtgcccctggagaccaccgagtgcatccagggccagggcgagggctaccggggcaccgtgaacaccatctggaacggcatcccctgccagcggtgggacagccagtacccccacgagcacgacatgacccccgagaacttcaagtgcaaggacctgcgggagaactactgccggaaccccgacggcagcgagagcccctggtgcttcaccaccgaccccaacatccgggtgggctactgcagccagatccccaactgcgacatgagccacggccaggactgctaccggggcaacggcaagaactacatgggcaacctgagccagacccggagcggcctgacctgcagcatgtgggacaagaacatggaggacctgcaccggcacatcttctgggagcccgacgccagcaagctgaacgagaactactgccggaaccccgacgacgacgcccacggcccctggtgctacaccggcaaccccctgatcccctgggactactgccccatcagccggtgcgagggcgacaccacccccaccatcgtgaacctggaccaccccgtgatcagctgcgccaagaccaagcagctgcgggtggtgaacggcatccccacccggaccaacatcggctggatggtgagcctgcggtaccggaacaagcacatctgcggcggcagcctgatcaaggagagctgggtgctgaccgcccggcagtgcttccccagccgggacctgaaggactacgaggcctggctgggcatccacgacgtgcacggccggggcgacgagaagtgcaagcaggtgctgaacgtgagccagctggtgtacggccccgagggcagcgacctggtgctgatgaagctggcccggcccgccgtgctggacgacttcgtgagcaccatcgacctgcccaactacggctgcaccatccccgagaagaccagctgcagcgtgtacggctggggctacaccggcctgatcaactacgacggcctgctgcgggtggcccacctgtacatcatgggcaacgagaagtgcagccagcaccaccggggcaaggtgaccctgaacgagagcgagatctgcgccggcgccgagaagatcggcagcggcccctgcgagggcgactacggcggccccctggtgtgcgagcagcacaagatgcggatggtgctgggcgtgatcgtgcccggccggggctgcgccatccccaaccggcccggcatcttcgtgcgggtggcctactacgccaagtggatccacaagatcatcctgacctacaaggtgccccagagctga

SEQ ID NO: 5 - DNA, 4955 bp, Artificial Sequence
  pVector-p42
ccaatgatcctgcaggcagctgcgcgctcgctcgctcactgaggccgcccgggcaaagcccgggcgtcgggcgacctttggtcgcccggcctcagtgagcgagcgagcgcgcagagagggagtggggttatcggcgcgccgcggccgcccatggactagtattatgcccagtacatgaccttatgggactttcctacttggcagtacatctacgtattagtcatcgctattaccatggtgatgcggttttggcagtacatcaatgggcgtggatagcggtttgactcacggggatttccaagtctccaccccattgacgtcaatgggagtttgttttggcaccaaaatcaacgggactttccaaaatgtcgtaacaactccgccccattgacgcaaatgggcggtaggcgtgtacggtgggaggtctatataagcagagctcgtttagtgaaccgtcagatcgcctggagacgccatccacgctgttttgacctccatagaagattctagagctagcgaattcgctagcggcccaggcggcccaccatgtgggtgaccaagctgctgcccgccctgctgctgcagcacgtgctgctgcacctgctgctgctgcccatcgccatcccctacgccgagggccagcggaagcggcggaacaccatccacgagttcaagaagagcgccaagaccaccctgatcaagatcgaccccgccctgaagatcaagaccaagaaggtgaacaccgccgaccagtgcgccaaccggtgcacccggaacaagggcctgcccttcacctgcaaggccttcgtgttcgacaaggcccggaagcagtgcctgtggttccccttcaacagcatgagcagcggcgtgaagaaggagttcggccacgagttcgacctgtacgagaacaaggactacatccggaactgcatcatcggcaagggccggagctacaagggcaccgtgagcatcaccaagagcggcatcaagtgccagccctggagcagcatgatcccccacgagcacagcttcctgcccagcagctaccggggcaaggacctgcaggagaactactgccggaacccccggggcgaggagggcggcccctggtgcttcaccagcaaccccgaggtgcggtacgaggtgtgcgacatcccccagtgcagcgaggtggagtgcatgacctgcaacggcgagagctaccggggcctgatggaccacaccgagagcggcaagatctgccagcggtgggaccaccagaccccccaccggcacaagttcctgcccgagcggtaccccgacaagggcttcgacgacaactactgccggaaccccgacggccagccccggccctggtgctacaccctggacccccacacccggtgggagtactgcgccatcaagacctgcgccgacaacaccatgaacgacaccgacgtgcccctggagaccaccgagtgcatccagggccagggcgagggctaccggggcaccgtgaacaccatctggaacggcatcccctgccagcggtgggacagccagtacccccacgagcacgacatgacccccgagaacttcaagtgcaaggacctgcgggagaactactgccggaaccccgacggcagcgagagcccctggtgcttcaccaccgaccccaacatccgggtgggctactgcagccagatccccaactgcgacatgagccacggccaggactgctaccggggcaacggcaagaactacatgggcaacctgagccagacccggagcggcctgacctgcagcatgtgggacaagaacatggaggacctgcaccggcacatcttctgggagcccgacgccagcaagctgaacgagaactactgccggaaccccgacgacgacgcccacggcccctggtgctacaccggcaaccccctgatcccctgggactactgccccatcagccggtgcgagggcgacaccacccccaccatcgtgaacctggaccaccccgtgatcagctgcgccaagaccaagcagctgcgggtggtgaacggcatccccacccggaccaacatcggctggatggtgagcctgcggtaccggaacaagcacatctgcggcggcagcctgatcaaggagagctgggtgctgaccgcccggcagtgcttccccagccgggacctgaaggactacgaggcctggctgggcatccacgacgtgcacggccggggcgacgagaagtgcaagcaggtgctgaacgtgagccagctggtgtacggccccgagggcagcgacctggtgctgatgaagctggcccggcccgccgtgctggacgacttcgtgagcaccatcgacctgcccaactacggctgcaccatccccgagaagaccagctgcagcgtgtacggctggggctacaccggcctgatcaactacgacggcctgctgcgggtggcccacctgtacatcatgggcaacgagaagtgcagccagcaccaccggggcaaggtgaccctgaacgagagcgagatctgcgccggcgccgagaagatcggcagcggcccctgcgagggcgactacggcggccccctggtgtgcgagcagcacaagatgcggatggtgctgggcgtgatcgtgcccggccggggctgcgccatccccaaccggcccggcatcttcgtgcgggtggcctactacgccaagtggatccacaagatcatcctgacctacaaggtgccccagagctgaggccaggccggccggatccatttaaatgatatcgatgatccagacatgataagatacattgatgagtttggacaaaccacaactagaatgcagtgaaaaaaatgctttatttgtgaaatttgtgatgctattgctttatttgtaaccattataagctgcaataaacaagttaacaacaacaattgcattcattttatgtttcaggttcagggggaggtgtgggaggttttttttaattaatctagagcggccgcaggaacccctagtgatggagttggccactccctctctgcgcgctcgctcgctcactgaggccgggcgaccaaaggtcgcccgacgcccgggctttgcccgggcggcctcagtgagcgagcgagcgcgcagctgcctgcaggatcggaaagaacatgtgagcaaaaggccagcaaaaggccaggaaccgtaaaaaggccgcgttgctggcgtttttccataggctccgcccccctgacgagcatcacaaaaatcgacgctcaagtcagaggtggcgaaacccgacaggactataaagataccaggcgtttccccctggaagctccctcgtgcgctctcctgttccgaccctgccgcttaccggatacctgtccgcctttctcccttcgggaagcgtggcgctttctcatagctcacgctgtaggtatctcagttcggtgtaggtcgttcgctccaagctgggctgtgtgcacgaaccccccgttcagcccgaccgctgcgccttatccggtaactatcgtcttgagtccaacccggtaagacacgacttatcgccactggcagcagccactggtaacaggattagcagagcgaggtatgtaggcggtgctacagagttcttgaagtggtggcctaactacggctacactagaagaacagtatttggtatctgcgctctgctgaagccagttaccttcggaaaaagagttggtagctcttgatccggcaaacaaaccaccgctggtagcggtggtttttttgtttgcaagcagcagattacgcgcagaaaaaaaggatctcaagaagatcctttgatcttttctacggggtctgacgctcagtggaacgaaaactcacgttaagggattttggtcatgagattatcaaaaaggatcttcacctagatccttttaaattaaaaatgaagttttaaatcaatctaaagtatatatgagtaaacttggtctgacagttaccaatgcttaatcagtgaggcacctatctcagcgatctgtctatttcgttcatccatagttgcctgactccccgtcgtgtagataactacgatacgggagggcttaccatctggccccagtgctgcaatgataccgcgagacccacgctcaccggctccagatttatcagcaataaaccagccagccggaagggccgagcgcagaagtggtcctgcaactttatccgcctccatccagtctattaattgttgccgggaagctagagtaagtagttcgccagttaatagtttgcgcaacgttgttgccattgctacaggcatcgtggtgtcacgctcgtcgtttggtatggcttcattcagctccggttcccaacgatcaaggcgagttacatgatcccccatgttgtgcaaaaaagcggttagctccttcggtcctccgatcgttgtcagaagtaagttggccgcagtgttatcactcatggttatggcagcactgcataattctcttactgtcatgccatccgtaagatgcttttctgtgactggtgagtactcaaccaagtcattctgagaatagtgtatgcggcgaccgagttgctcttgcccggcgtcaatacgggataataccgcgccacatagcagaactttaaaagtgctcatcattggaaaacgttcttcggggcgaaaactctcaaggatcttaccgctgttgagatccagttcgatgtaacccactcgtgcacccaactgatcttcagcatcttttactttcaccagcgtttctgggtgagcaaaaacaggaaggcaaaatgccgcaaaaaagggaataagggcgacacggaaatgttgaatactcatactcttcctttttcaatattattgaagcatttatcagggttattgtctcatgagcggatacatatttgaatgtatttagaaaaataaacaaataggggttccgcgcacatttccccgaaaagtgccacctgacgtc

SEQ ID NO: 6 - DNA, 5788 bp, Artificial Sequence
  pVector-p13
ccaatgatcctgcaggcagctgcgcgctcgctcgctcactgaggccgcccgggcaaagcccgggcgtcgggcgacctttggtcgcccggcctcagtgagcgagcgagcgcgcagagagggagtggccaactccatcactaggggttcctgcggccgcccatggactagtattaatagtaatcaattacggggtcattagttcatagcccatatatggagttccgcgttacataacttacggtaaatggcccgcctggctgaccgcccaacgacccccgcccattgacgtcaataatgacgtatgttcccatagtaacgccaatagggactttccattgacgtcaatgggtggagtatttacggtaaactgcccacttggcagtacatcaagtgtatcatatgccaagtacgccccctattgacgtcaatgacggtaaatggcccgcctggcattatgcccagtacatgaccttatgggactttcctacttggcagtacatctacgtattagtcatcgctattaccatggtgatgcggttttggcagtacatcaatgggcgtggatagcggtttgactcacggggatttccaagtctccaccccattgacgtcaatgggagtttgttttggcaccaaaatcaacgggactttccaaaatgtcgtaacaactccgccccattgacgcaaatgggcggtaggcgtgtacggtgggaggtctatataagcagagctcgtttagtgaaccgtcagatcgaattcgctagcggcccaggcggcccaccatgtgggtgaccaagctgctgcccgccctgctgctgcagcacgtgctgctgcacctgctgctgctgcccatcgccatcccctacgccgagggccagcggaagcggcggaacaccatccacgagttcaagaagagcgccaagaccaccctgatcaagatcgaccccgccctgaagatcaagaccaagaaggtgaacaccgccgaccagtgcgccaaccggtgcacccggaacaagggcctgcccttcacctgcaaggccttcgtgttcgacaaggcccggaagcagtgcctgtggttccccttcaacagcatgagcagcggcgtgaagaaggagttcggccacgagttcgacctgtacgagaacaaggactacatccggaactgcatcatcggcaagggccggagctacaagggcaccgtgagcatcaccaagagcggcatcaagtgccagccctggagcagcatgatcccccacgagcacagcttcctgcccagcagctaccggggcaaggacctgcaggagaactactgccggaacccccggggcgaggagggcggcccctggtgcttcaccagcaaccccgaggtgcggtacgaggtgtgcgacatcccccagtgcagcgaggtggagtgcatgacctgcaacggcgagagctaccggggcctgatggaccacaccgagagcggcaagatctgccagcggtgggaccaccagaccccccaccggcacaagttcctgcccgagcggtaccccgacaagggcttcgacgacaactactgccggaaccccgacggccagccccggccctggtgctacaccctggacccccacacccggtgggagtactgcgccatcaagacctgcgccgacaacaccatgaacgacaccgacgtgcccctggagaccaccgagtgcatccagggccagggcgagggctaccggggcaccgtgaacaccatctggaacggcatcccctgccagcggtgggacagccagtacccccacgagcacgacatgacccccgagaacttcaagtgcaaggacctgcgggagaactactgccggaaccccgacggcagcgagagcccctggtgcttcaccaccgaccccaacatccgggtgggctactgcagccagatccccaactgcgacatgagccacggccaggactgctaccggggcaacggcaagaactacatgggcaacctgagccagacccggagcggcctgacctgcagcatgtgggacaagaacatggaggacctgcaccggcacatcttctgggagcccgacgccagcaagctgaacgagaactactgccggaaccccgacgacgacgcccacggcccctggtgctacaccggcaaccccctgatcccctgggactactgccccatcagccggtgcgagggcgacaccacccccaccatcgtgaacctggaccaccccgtgatcagctgcgccaagaccaagcagctgcgggtggtgaacggcatccccacccggaccaacatcggctggatggtgagcctgcggtaccggaacaagcacatctgcggcggcagcctgatcaaggagagctgggtgctgaccgcccggcagtgcttccccagccgggacctgaaggactacgaggcctggctgggcatccacgacgtgcacggccggggcgacgagaagtgcaagcaggtgctgaacgtgagccagctggtgtacggccccgagggcagcgacctggtgctgatgaagctggcccggcccgccgtgctggacgacttcgtgagcaccatcgacctgcccaactacggctgcaccatccccgagaagaccagctgcagcgtgtacggctggggctacaccggcctgatcaactacgacggcctgctgcgggtggcccacctgtacatcatgggcaacgagaagtgcagccagcaccaccggggcaaggtgaccctgaacgagagcgagatctgcgccggcgccgagaagatcggcagcggcccctgcgagggcgactacggcggccccctggtgtgcgagcagcacaagatgcggatggtgctgggcgtgatcgtgcccggccggggctgcgccatccccaaccggcccggcatcttcgtgcgggtggcctactacgccaagtggatccacaagatcatcctgacctacaaggtgccccagagctgaggccaggccggccggatccatcgataatcaacctctggattacaaaatttgtgaaagattgactgatattcttaactatgttgctccttttacgctgtgtggatatgctgctttaatgcctctgtatcatgctattgcttcccgtacggctttcgttttctcctccttgtataaatcctggttgctgtctctttatgaggagttgtggcccgttgtccgtcaacgtggcgtggtgtgctctgtgtttgctgacgcaacccccactggctggggcattgccaccacctgtcaactcctttctgggactttcgctttccccctcccgatcgccacggcagaactcatcgccgcctgccttgcccgctgctggacaggggctaggttgctgggcactgataattccgtggtgttgtcggggaaatcatcgtcctttccttggctgctcgcctgtgttgccaactggatcctgcgcgggacgtccttctgctacgtcccttcggctctcaatccagcggacctcccttcccgaggccttctgccggttctgcggcctctcccgcgtcttcgctttcggcctccgacgagtcggatctccctttgggccgcctccccgcctatttaaatgatatcgatgatccagacatgataagatacattgatgagtttggacaaaccacaactagaatgcagtgaaaaaaatgctttatttgtgaaatttgtgatgctattgctttatttgtaaccattataagctgcaataaacaagttaacaacaacaattgcattcattttatgtttcaggttcagggggaggtgtgggaggttttttttaattaatctagagcggccgcaggaacccctagtgatggagttggccactccctctctgcgcgctcgctcgctcactgaggccgggcgaccaaaggtcgcccgacgcccgggctttgcccgggcggcctcagtgagcgagcgagcgcgcagctgcctgcaggatcggaaagaacatgtgagcaaaaggccagcaaaaggccaggaaccgtaaaaaggccgcgttgctggcgtttttccataggctccgcccccctgacgagcatcacaaaaatcgacgctcaagtcagaggtggcgaaacccgacaggactataaagataccaggcgtttccccctggaagctccctcgtgcgctctcctgttccgaccctgccgcttaccggatacctgtccgcctttctcccttcgggaagcgtggcgctttctcatagctcacgctgtaggtatctcagttcggtgtaggtcgttcgctccaagctgggctgtgtgcacgaaccccccgttcagcccgaccgctgcgccttatccggtaactatcgtcttgagtccaacccggtaagacacgacttatcgccactggcagcagccactggtaacaggattagcagagcgaggtatgtaggcggtgctacagagttcttgaagtggtggcctaactacggctacactagaagaacagtatttggtatctgcgctctgctgaagccagttaccttcggaaaaagagttggtagctcttgatccggcaaacaaaccaccgctggtagcggtggtttttttgtttgcaagcagcagattacgcgcagaaaaaaaggatctcaagaagatcctttgatcttttctacggggtctgacgctcagtggaacgaaaactcacgttaagggattttggtcatgagattatcaaaaaggatcttcacctagatccttttaaattaaaaatgaagttttaaatcaatctaaagtatatatgagtaaacttggtctgacagttaccaatgcttaatcagtgaggcacctatctcagcgatctgtctatttcgttcatccatagttgcctgactccccgtcgtgtagataactacgatacgggagggcttaccatctggccccagtgctgcaatgataccgcgagacccacgctcaccggctccagatttatcagcaataaaccagccagccggaagggccgagcgcagaagtggtcctgcaactttatccgcctccatccagtctattaattgttgccgggaagctagagtaagtagttcgccagttaatagtttgcgcaacgttgttgccattgctacaggcatcgtggtgtcacgctcgtcgtttggtatggcttcattcagctccggttcccaacgatcaaggcgagttacatgatcccccatgttgtgcaaaaaagcggttagctccttcggtcctccgatcgttgtcagaagtaagttggccgcagtgttatcactcatggttatggcagcactgcataattctcttactgtcatgccatccgtaagatgcttttctgtgactggtgagtactcaaccaagtcattctgagaatagtgtatgcggcgaccgagttgctcttgcccggcgtcaatacgggataataccgcgccacatagcagaactttaaaagtgctcatcattggaaaacgttcttcggggcgaaaactctcaaggatcttaccgctgttgagatccagttcgatgtaacccactcgtgcacccaactgatcttcagcatcttttactttcaccagcgtttctgggtgagcaaaaacaggaaggcaaaatgccgcaaaaaagggaataagggcgacacggaaatgttgaatactcatactcttcctttttcaatattattgaagcatttatcagggttattgtctcatgagcggatacatatttgaatgtatttagaaaaataaacaaataggggttccgcgcacatttccccgaaaagtgccacctgacgtc

SEQ ID NO: 7 - DNA, 592 bp, Artificial Sequence
  Woodchuck Hepatitis Virus Post-transcriptional Regulatory Element(WPRE)-mut6 sequence
taatcaacctctggattacaaaatttgtgaaagattgactgatattcttaactatgttgctccttttacgctgtgtggatatgctgctttaatgcctctgtatcatgctattgcttcccgtacggctttcgttttctcctccttgtataaatcctggttgctgtctctttatgaggagttgtggcccgttgtccgtcaacgtggcgtggtgtgctctgtgtttgctgacgcaacccccactggctggggcattgccaccacctgtcaactcctttctgggactttcgctttccccctcccgatcgccacggcagaactcatcgccgcctgccttgcccgctgctggacaggggctaggttgctgggcactgataattccgtggtgttgtcggggaaatcatcgtcctttccttggctgctcgcctgtgttgccaactggatcctgcgcgggacgtccttctgctacgtcccttcggctctcaatccagcggacctcccttcccgaggccttctgccggttctgcggcctctcccgcgtcttcgctttcggcctccgacgagtcggatctccctttgggccgcctccccgcct

SEQ ID NO: 8 - DNA, 20 bp, Artificial Sequence
  Forward primer for optHGF
taccggaacaagcacatctg

SEQ ID NO: 9 - DNA, 18 bp, Artificial Sequence
  Reverse primer for optHGF
ttcatcagcaccaggtcg

SEQ ID NO: 10 - DNA, 20 bp, Artificial Sequence
  Forward primer for GAPDH
catcactgccacccagaaga

SEQ ID NO: 11 - DNA, 15 bp, Artificial Sequence
  Reverse primer for GAPDH
atgttctgggcagcc

SEQ ID NO: 12 - DNA, 121 bp, Artificial Sequence
  Mutant-type ITR sequence
ctgcgcgctcgctcgctcactgaggccgcccgggcaaagcccgggcgtcgggcgacctttggtcgcccggcctcagtgagcgagcgagcgcgcagagagggagtggggttatcggcgcgcc

SEQ ID NO: 13 - DNA, 130 bp, Artificial Sequence
  Non mutant-type 3'-ITR sequence
aggaacccctagtgatggagttggccactccctctctgcgcgctcgctcgctcactgaggccgggcgaccaaaggtcgcccgacgcccgggctttgcccgggcggcctcagtgagcgagcgagcgcgcag

SEQ ID NO: 14 - DNA, 130 bp, Artificial Sequence
  Non mutant-type 5'-ITR sequence
ctgcgcgctcgctcgctcactgaggccgcccgggcaaagcccgggcgtcgggcgacctttggtcgcccggcctcagtgagcgagcgagcgcgcagagagggagtggccaactccatcactaggggttcct

SEQ ID NO: 15 - DNA, 196 bp, Simian virus
gatccagacatgataagatacattgatgagtttggacaaaccacaactagaatgcagtgaaaaaaatgctttatttgtgaaatttgtgatgctattgctttatttgtaaccattataagctgcaataaacaagttaacaacaacaattgcattcattttatgtttcaggttcagggggaggtgtgggaggtttttt

SEQ ID NO: 16 - DNA, 2424 bp, Artificial Sequence
  pVector (empty vector)
ccaatgatcctgcaggcagctgcgcgctcgctcgctcactgaggccgcccgggcaaagcccgggcgtcgggcgacctttggtcgcccggcctcagtgagcgagcgagcgcgcagagagggagtggggttatcggcgcgccgcggccgcccatggactagtttctagagctagcgaattcgctagcggcccaggcggcccaccggccaggccggccggatccatttaaatgatatcgatgatccagacatgataagatacattgatgagtttggacaaaccacaactagaatgcagtgaaaaaaatgctttatttgtgaaatttgtgatgctattgctttatttgtaaccattataagctgcaataaacaagttaacaacaacaattgcattcattttatgtttcaggttcagggggaggtgtgggaggttttttttaattaatctagagcggccgcaggaacccctagtgatggagttggccactccctctctgcgcgctcgctcgctcactgaggccgggcgaccaaaggtcgcccgacgcccgggctttgcccgggcggcctcagtgagcgagcgagcgcgcagctgcctgcaggatcggaaagaacatgtgagcaaaaggccagcaaaaggccaggaaccgtaaaaaggccgcgttgctggcgtttttccataggctccgcccccctgacgagcatcacaaaaatcgacgctcaagtcagaggtggcgaaacccgacaggactataaagataccaggcgtttccccctggaagctccctcgtgcgctctcctgttccgaccctgccgcttaccggatacctgtccgcctttctcccttcgggaagcgtggcgctttctcatagctcacgctgtaggtatctcagttcggtgtaggtcgttcgctccaagctgggctgtgtgcacgaaccccccgttcagcccgaccgctgcgccttatccggtaactatcgtcttgagtccaacccggtaagacacgacttatcgccactggcagcagccactggtaacaggattagcagagcgaggtatgtaggcggtgctacagagttcttgaagtggtggcctaactacggctacactagaagaacagtatttggtatctgcgctctgctgaagccagttaccttcggaaaaagagttggtagctcttgatccggcaaacaaaccaccgctggtagcggtggtttttttgtttgcaagcagcagattacgcgcagaaaaaaaggatctcaagaagatcctttgatcttttctacggggtctgacgctcagtggaacgaaaactcacgttaagggattttggtcatgagattatcaaaaaggatcttcacctagatccttttaaattaaaaatgaagttttaaatcaatctaaagtatatatgagtaaacttggtctgacagttaccaatgcttaatcagtgaggcacctatctcagcgatctgtctatttcgttcatccatagttgcctgactccccgtcgtgtagataactacgatacgggagggcttaccatctggccccagtgctgcaatgataccgcgagacccacgctcaccggctccagatttatcagcaataaaccagccagccggaagggccgagcgcagaagtggtcctgcaactttatccgcctccatccagtctattaattgttgccgggaagctagagtaagtagttcgccagttaatagtttgcgcaacgttgttgccattgctacaggcatcgtggtgtcacgctcgtcgtttggtatggcttcattcagctccggttcccaacgatcaaggcgagttacatgatcccccatgttgtgcaaaaaagcggttagctccttcggtcctccgatcgttgtcagaagtaagttggccgcagtgttatcactcatggttatggcagcactgcataattctcttactgtcatgccatccgtaagatgcttttctgtgactggtgagtactcaaccaagtcattctgagaatagtgtatgcggcgaccgagttgctcttgcccggcgtcaatacgggataataccgcgccacatagcagaactttaaaagtgctcatcattggaaaacgttcttcggggcgaaaactctcaaggatcttaccgctgttgagatccagttcgatgtaacccactcgtgcacccaactgatcttcagcatcttttactttcaccagcgtttctgggtgagcaaaaacaggaaggcaaaatgccgcaaaaaagggaataagggcgacacggaaatgttgaatactcatactcttcctttttcaatattattgaagcatttatcagggttattgtctcatgagcggatacatatttgaatgtatttagaaaaataaacaaataggggttccgcgcacatttccccgaaaagtgccacctgacgtc